European Patent Specification EP 3 209 692 B1, published May 22, 2024. Title: METHODS AND PRODUCTS FOR MODULATING MICROBIOTA COMPOSITION FOR IMPROVING THE EFFICACY OF A CANCER TREATMENT WITH AN IMMUNE CHECKPOINT BLOCKER. Applicant: INSTITUT GUSTAVE ROUSSY ZITVOGEL, Laurence VETIZOU, Marie LEPAGE, Patricia. The sequence listing filed with the application follows.

SEQUENCE LISTING (10 sequences)

SEQ ID NO: 1 - DNA, 20 bp, Artificial Sequence
  primers
tgattccgcatggtttcatt

SEQ ID NO: 2 - DNA, 20 bp, Artificial Sequence
  Primers
cgacccatagagccttcatc

SEQ ID NO: 3 - DNA, 25 bp, Artificial Sequence
  Primers
ggtagtccacacagtaaacgatgaa

SEQ ID NO: 4 - DNA, 22 bp, Artificial Sequence
  Primers
cccgtcaattcctttgagtttc

SEQ ID NO: 5 - DNA, 23 bp, Artificial Sequence
  Primers
tcttccgcatggtagaactatta

SEQ ID NO: 6 - DNA, 22 bp, Artificial Sequence
  Primers
accgtgtctcagttccaatgtg

SEQ ID NO: 7 - DNA, 21 bp, Artificial Sequence
  Primers
tgcctatcagagggggataac

SEQ ID NO: 8 - DNA, 21 bp, Artificial Sequence
  Primers
gcaaatattcccatgcgggat

SEQ ID NO: 9 - DNA, 21 bp, Artificial Sequence
  Primers
actcctacgggaggcagcagt

SEQ ID NO: 10 - DNA, 18 bp, Artificial Sequence
  Primers
attaccgcggctgctggc